European Patent Application EP 4 289 866 A2, published December 13, 2023. Title: Anti-PD-1 antibody and use thereof. Applicant: GENUV Inc. The sequence listing filed with the application follows.

SEQUENCE LISTING (84 sequences)

SEQ ID NO: 1 - protein, 5 aa, Artificial Sequence
  HCDR1 aa
GYWMH

SEQ ID NO: 2 - DNA, 15 bp, Artificial Sequence
  HCDR1 nucleotide
ggctactggatgcac

SEQ ID NO: 3 - protein, 17 aa, Artificial Sequence
  HCDR2 aa
MIHPNSDTTTYNEKFKN

SEQ ID NO: 4 - DNA, 51 bp, Artificial Sequence
  HCDR2 nucleotide
atgattcatcctaacagtgatactactacctacaatgagaagttcaaaaac

SEQ ID NO: 5 - protein, 9 aa, Artificial Sequence
  HCDR3 aa
TDQAAWFAF

SEQ ID NO: 6 - DNA, 27 bp, Artificial Sequence
  HCDR3 nucleotide
acagatcaggccgcctggtttgctttc

SEQ ID NO: 7 - protein, 16 aa, Artificial Sequence
  LCDR1 aa
RSSQNIVHSNGDTYLE

SEQ ID NO: 8 - DNA, 48 bp, Artificial Sequence
  LCDR1 nucleotide
agatctagtcagaacattgtacatagtaatggagacacctatttagaa

SEQ ID NO: 9 - protein, 7 aa, Artificial Sequence
  LCDR2 aa
KVSKRFS

SEQ ID NO: 10 - DNA, 21 bp, Artificial Sequence
  LCDR2 nucleotide
aaagtttccaagcgattttct

SEQ ID NO: 11 - protein, 9 aa, Artificial Sequence
  LCDR3 aa
FQGSHVPWT

SEQ ID NO: 12 - DNA, 27 bp, Artificial Sequence
  LCDR3 nucleotide
tttcaaggttcacatgttccgtggacg

SEQ ID NO: 13 - protein, 118 aa, Artificial Sequence
  HCVR aa
EVQLQQSGAELVKPGASVKLSCKASGYTFTGYWMHWVKQRPGQGLEWIGMIHPNSDTTTYNEKFKNRATLTVDKSSGTAYMQLSSLTSEDSAVYYCTGTDQAAWFAFWGQGTLVTVSA

SEQ ID NO: 14 - DNA, 354 bp, Artificial Sequence
  HCVR nucleotide
gaggtccagctgcagcagtctggggctgagctggttaagcctggggcttcagtgaagctgtcctgcaaggcttctggctacactttcaccggctactggatgcactgggtgaagcagaggcctggacaaggccttgagtggattggaatgattcatcctaacagtgatactactacctacaatgagaagttcaaaaacagggccacactgactgtagacaaatcctccggcacagcctacatgcaactcagcagcctgacatctgaggactctgcggtctattactgtacagggacagatcaggccgcctggtttgctttctggggccaagggactctggtcactgtctctgca

SEQ ID NO: 15 - protein, 112 aa, Artificial Sequence
  LCVR aa
DIVLTQTPLSLPVSLGDQASISCRSSQNIVHSNGDTYLEWYLQKPGQSPKLLIYKVSKRFSGVPDRFSGSGSGTDFTLKISRVEAEDLGVYYCFQGSHVPWTFGGGTKLEIK

SEQ ID NO: 16 - DNA, 336 bp, Artificial Sequence
  LCVR nucleotide
gatattgtgctgacacaaactccactctccctgcctgtcagtcttggagatcaagcctccatctcttgcagatctagtcagaacattgtacatagtaatggagacacctatttagaatggtacctgcagaaaccaggccagtctccaaagctcctgatctacaaagtttccaagcgattttctggggtcccagacaggttcagtggcagtggatcagggacagatttcacactcaagatcagcagagtggaggctgaggatctgggagtttattactgctttcaaggttcacatgttccgtggacgttcggtggaggcaccaagctggaaatcaaa

SEQ ID NO: 17 - protein, 30 aa, Artificial Sequence
  HFR1 aa
EVQLQQSGAELVKPGASVKLSCKASGYTFT

SEQ ID NO: 18 - DNA, 90 bp, Artificial Sequence
  HFR1 nucleotide
gaggtccagctgcagcagtctggggctgagctggttaagcctggggcttcagtgaagctgtcctgcaaggcttctggctacactttcacc

SEQ ID NO: 19 - protein, 14 aa, Artificial Sequence
  HFR2 aa
WVKQRPGQGLEWIG

SEQ ID NO: 20 - DNA, 42 bp, Artificial Sequence
  HFR2 nucleotide
tgggtgaagcagaggcctggacaaggccttgagtggattgga

SEQ ID NO: 21 - protein, 32 aa, Artificial Sequence
  HFR3 aa
RATLTVDKSSGTAYMQLSSLTSEDSAVYYCTG

SEQ ID NO: 22 - DNA, 96 bp, Artificial Sequence
  HFR3 nucleotide
agggccacactgactgtagacaaatcctccggcacagcctacatgcaactcagcagcctgacatctgaggactctgcggtctattactgtacaggg

SEQ ID NO: 23 - protein, 11 aa, Artificial Sequence
  HFR4 aa
WGQGTLVTVSA

SEQ ID NO: 24 - DNA, 33 bp, Artificial Sequence
  HFR4 nucleotide
tggggccaagggactctggtcactgtctctgca

SEQ ID NO: 25 - protein, 23 aa, Artificial Sequence
  LFR1 aa
DIVLTQTPLSLPVSLGDQASISC

SEQ ID NO: 26 - DNA, 69 bp, Artificial Sequence
  LFR1 nucleotide
gatattgtgctgacacaaactccactctccctgcctgtcagtcttggagatcaagcctccatctcttgc

SEQ ID NO: 27 - protein, 15 aa, Artificial Sequence
  LFR2 aa
WYLQKPGQSPKLLIY

SEQ ID NO: 28 - DNA, 45 bp, Artificial Sequence
  LFR2 nucleotide
tggtacctgcagaaaccaggccagtctccaaagctcctgatctac

SEQ ID NO: 29 - protein, 32 aa, Artificial Sequence
  LFR3 aa
GVPDRFSGSGSGTDFTLKISRVEAEDLGVYYC

SEQ ID NO: 30 - DNA, 96 bp, Artificial Sequence
  LFR3 nucleotide
ggggtcccagacaggttcagtggcagtggatcagggacagatttcacactcaagatcagcagagtggaggctgaggatctgggagtttattactgc

SEQ ID NO: 31 - protein, 10 aa, Artificial Sequence
  LFR4 aa
FGGGTKLEIK

SEQ ID NO: 32 - DNA, 30 bp, Artificial Sequence
  LFR4 nucleotide
ttcggtggaggcaccaagctggaaatcaaa

SEQ ID NO: 33 - DNA, 31 bp, Artificial Sequence
  MH1 primer
aatttgctagcsargtnmagctgsagsagtc

SEQ ID NO: 34 - DNA, 34 bp, Artificial Sequence
  MH2 primer
aatttgctagcsargtnmagctgsagsagtcwgg

SEQ ID NO: 35 - DNA, 38 bp, Artificial Sequence
  IgG1 primer
aatttggatccatagacagatgggggtgtcgttttggc

SEQ ID NO: 36 - DNA, 34 bp, Artificial Sequence
  MK primer
aattggatccaggggccagtggatagactgatgg

SEQ ID NO: 37 - DNA, 34 bp, Artificial Sequence
  CK primer
aatttgcggccgcggatacagttggtgcagcatc

SEQ ID NO: 38 - DNA, 981 bp, Artificial Sequence
  Human IgG4 CH
gctagcaccaagggcccatcggtcttccccctggcgccctgctccaggagcacctccgagagcacagccgccctgggctgcctggtcaaggactacttccccgaacccgtgacggtgtcgtggaactcaggcgccctgaccagcggcgtgcacaccttcccggctgtcctacagtcctcaggactctactccctcagcagcgtggtgaccgtgccctccagcagcttgggcacgaagacctacacctgcaacgtagatcacaagcccagcaacaccaaggtggacaagagagttgagtccaaatatggtcccccatgcccaccatgcccagcacctgagttcctggggggaccatcagtcttcctgttccccccaaaacccaaggacactctcatgatctcccggacccctgaggtcacgtgcgtggtggtggacgtgagccaggaagaccccgaggtccagttcaactggtacgtggatggcgtggaggtgcataatgccaagacaaagccgcgggaggagcagttcaacagcacgtaccgtgtggtcagcgtcctcaccgtcctgcaccaggactggctgaacggcaaggagtacaagtgcaaggtctccaacaaaggcctcccgtcctccatcgagaaaaccatctccaaagccaaagggcagccccgagagccacaggtgtacaccctgcccccatcccaggaggagatgaccaagaaccaggtcagcctgacctgcctggtcaaaggcttctaccccagcgacatcgccgtggagtgggagagcaatgggcagccggagaacaactacaagaccacgcctcccgtgctggactccgacggctccttcttcctctacagcaggctaaccgtggacaagagcaggtggcaggaggggaatgtcttctcatgctccgtgatgcatgaggctctgcacaaccactacacacagaagagcctctccctgtctccgggtaaa

SEQ ID NO: 39 - protein, 327 aa, Artificial Sequence
  Human IgG4 CH
ASTKGPSVFPLAPCSRSTSESTAALGCLVKDYFPEPVTVSWNSGALTSGVHTFPAVLQSSGLYSLSSVVTVPSSSLGTKTYTCNVDHKPSNTKVDKRVESKYGPPCPPCPAPEFLGGPSVFLFPPKPKDTLMISRTPEVTCVVVDVSQEDPEVQFNWYVDGVEVHNAKTKPREEQFNSTYRVVSVLTVLHQDWLNGKEYKCKVSNKGLPSSIEKTISKAKGQPREPQVYTLPPSQEEMTKNQVSLTCLVKGFYPSDIAVEWESNGQPENNYKTTPPVLDSDGSFFLYSRLTVDKSRWQEGNVFSCSVMHEALHNHYTQKSLSLSPGK

SEQ ID NO: 40 - DNA, 321 bp, Artificial Sequence
  Human IgG4 Ckappa
cgtacggtggctgcaccatctgtcttcatcttcccgccatctgatgagcagttgaaatctggaactgcctctgttgtgtgcctgctgaataacttctatcccagagaggccaaagtacagtggaaggtggataacgccctccaatcgggtaactcccaggagagtgtcacagagcaggacagcaaggacagcacctacagcctcagcagcaccctgacgctgagcaaagcagactacgagaaacacaaagtctacgcctgcgaagtcacccatcagggcctgagctcgcccgtcacaaagagcttcaacaggggagagtgt

SEQ ID NO: 41 - protein, 107 aa, Artificial Sequence [sequence omitted]

SEQ ID NO: 42 - DNA, 1341 bp, Artificial Sequence
  Humanized antibody, 1G1-h61 heavy chain nucleotides
caagttcagctggtgcagagcggcgccgaggtgaagaagcctggagccagcgtgaaagtgtcctgcaaggcctctggctacacctttacaggctactggatgcactgggtgcggcaggcccctggacagggcctggaatggatgggcatgatccaccccaacagcgacaccacaacctacaacgagaagttcaagaatagagtgaccatgacaagagataccagcatcagcaccgcctacatggaactgagcagactgcggtccgatgacacagctgtgtactattgtgccggcaccgaccaggccgcttggttcgccttctgggggcagggcaccacagtcaccgtgagctctgccagcaccaagggcccttccgtgtttcccctggccccttgctcccggtccacatctgagagcaccgccgccctgggctgtctggtgaaggactacttcccagagcccgtgaccgtgagctggaacagcggcgccctgacaagcggcgtgcacacatttcccgccgtgctgcagagctccggcctgtactccctgtctagcgtggtgacagtgccttcctctagcctgggcaccaagacatatacctgtaacgtggaccacaagccaagcaataccaaggtggataagcgggtggagtctaagtacggccctccttgccctagctgtcctgctccagagtttctgggcggcccttccgtgttcctgtttccacccaaaccaaaggacacactgatgatctctagaacaccagaggtgacctgcgtggtggtggacgtgagccaggaggatcccgaggtgcagttcaactggtacgtggatggcgtggaggtgcacaatgccaagaccaagccaagagaggagcagtttaactctacatacagggtggtgagcgtgctgaccgtgctgcaccaggattggctcaacggcaaggagtataagtgcaaggtgtccaataagggcctgccctcctctatcgagaagacaatctctaaggctaagggccagccaagagagcctcaggtgtacaccctgcctccaagccaggaggagatgacaaagaaccaggtgtccctgacatgtctggtgaagggcttctatccctccgacatcgccgtggagtgggagtctaatggccagcctgagaacaattacaagaccacaccccctgtgctggactctgatggcagcttctttctgtattccaggctgaccgtggataagtctcggtggcaggagggcaacgtgttcagctgctctgtgatgcacgaagccctgcataatcactatactcagaaaagtctgtcactgtcactgggaaagtgataa

SEQ ID NO: 43 - protein, 445 aa, Artificial Sequence
  Humanized antibody, 1G1-h61 heavy chain amino acids
QVQLVQSGAEVKKPGASVKVSCKASGYTFTGYWMHWVRQAPGQGLEWMGMIHPNSDTTTYNEKFKNRVTMTRDTSISTAYMELSRLRSDDTAVYYCAGTDQAAWFAFWGQGTTVTVSSASTKGPSVFPLAPCSRSTSESTAALGCLVKDYFPEPVTVSWNSGALTSGVHTFPAVLQSSGLYSLSSVVTVPSSSLGTKTYTCNVDHKPSNTKVDKRVESKYGPPCPSCPAPEFLGGPSVFLFPPKPKDTLMISRTPEVTCVVVDVSQEDPEVQFNWYVDGVEVHNAKTKPREEQFNSTYRVVSVLTVLHQDWLNGKEYKCKVSNKGLPSSIEKTISKAKGQPREPQVYTLPPSQEEMTKNQVSLTCLVKGFYPSDIAVEWESNGQPENNYKTTPPVLDSDGSFFLYSRLTVDKSRWQEGNVFSCSVMHEALHNHYTQKSLSLSLGK

SEQ ID NO: 44 - DNA, 1341 bp, Artificial Sequence
  Humanized antibody, 1G1-h68 heavy chain nucleotides
caagttcagctggtgcagagcggcgccgaggtgaagaagcctggagccagcgtgaaagtgtcctgcaaggcctctggctacacctttacaggctactggatgcactgggtgcggcaggcccctggacagggcctggaatggatcggcatgatccaccccaacagcgacaccacaacctacaacgagaagttcaagaatagagtgaccatgacaagagataccagcatcagcaccgcctacatggaactgagcagactgcggtccgatgacacagctgtgtactattgtaccggcaccgaccaggccgcttggttcgccttctgggggcagggcaccacagtcaccgtgagctctgccagcaccaagggcccttccgtgtttcccctggccccttgctcccggtccacatctgagagcaccgccgccctgggctgtctggtgaaggactacttcccagagcccgtgaccgtgagctggaacagcggcgccctgacaagcggcgtgcacacatttcccgccgtgctgcagagctccggcctgtactccctgtctagcgtggtgacagtgccttcctctagcctgggcaccaagacatatacctgtaacgtggaccacaagccaagcaataccaaggtggataagcgggtggagtctaagtacggccctccttgccctagctgtcctgctccagagtttctgggcggcccttccgtgttcctgtttccacccaaaccaaaggacacactgatgatctctagaacaccagaggtgacctgcgtggtggtggacgtgagccaggaggatcccgaggtgcagttcaactggtacgtggatggcgtggaggtgcacaatgccaagaccaagccaagagaggagcagtttaactctacatacagggtggtgagcgtgctgaccgtgctgcaccaggattggctcaacggcaaggagtataagtgcaaggtgtccaataagggcctgccctcctctatcgagaagacaatctctaaggctaagggccagccaagagagcctcaggtgtacaccctgcctccaagccaggaggagatgacaaagaaccaggtgtccctgacatgtctggtgaagggcttctatccctccgacatcgccgtggagtgggagtctaatggccagcctgagaacaattacaagaccacaccccctgtgctggactctgatggcagcttctttctgtattccaggctgaccgtggataagtctcggtggcaggagggcaacgtgttcagctgctctgtgatgcacgaagccctgcataatcactatactcagaaaagtctgtcactgtcactgggaaagtgataa

SEQ ID NO: 45 - protein, 445 aa, Artificial Sequence
  Humanized antibody, 1G1-h68 heavy chain amino acids
QVQLVQSGAEVKKPGASVKVSCKASGYTFTGYWMHWVRQAPGQGLEWIGMIHPNSDTTTYNEKFKNRVTMTRDTSISTAYMELSRLRSDDTAVYYCTGTDQAAWFAFWGQGTTVTVSSASTKGPSVFPLAPCSRSTSESTAALGCLVKDYFPEPVTVSWNSGALTSGVHTFPAVLQSSGLYSLSSVVTVPSSSLGTKTYTCNVDHKPSNTKVDKRVESKYGPPCPSCPAPEFLGGPSVFLFPPKPKDTLMISRTPEVTCVVVDVSQEDPEVQFNWYVDGVEVHNAKTKPREEQFNSTYRVVSVLTVLHQDWLNGKEYKCKVSNKGLPSSIEKTISKAKGQPREPQVYTLPPSQEEMTKNQVSLTCLVKGFYPSDIAVEWESNGQPENNYKTTPPVLDSDGSFFLYSRLTVDKSRWQEGNVFSCSVMHEALHNHYTQKSLSLSLGK

SEQ ID NO: 46 - DNA, 1341 bp, Artificial Sequence
  Humanized antibody, 1G1-h70 heavy chain nucleotides
caagttcagctggtgcagagcggcgccgaggtgaagaagcctggagccagcgtgaaagtgtcctgcaaggcctctggctacacctttacaggctactggatgcactgggtgcggcaggcccctggacagggcctggaatggatcggcatgatccaccccaacagcgacaccacaacctacaacgagaagttcaagaatagagtgaccatgacaagagataccagcatcagcaccgcctacatggaactgagcagactgcggtccgatgacacagctgtgtactattgtgccggcaccgaccaggccgcttggttcgccttctgggggcagggcaccacagtcaccgtgagctctgccagcaccaagggcccttccgtgtttcccctggccccttgctcccggtccacatctgagagcaccgccgccctgggctgtctggtgaaggactacttcccagagcccgtgaccgtgagctggaacagcggcgccctgacaagcggcgtgcacacatttcccgccgtgctgcagagctccggcctgtactccctgtctagcgtggtgacagtgccttcctctagcctgggcaccaagacatatacctgtaacgtggaccacaagccaagcaataccaaggtggataagcgggtggagtctaagtacggccctccttgccctagctgtcctgctccagagtttctgggcggcccttccgtgttcctgtttccacccaaaccaaaggacacactgatgatctctagaacaccagaggtgacctgcgtggtggtggacgtgagccaggaggatcccgaggtgcagttcaactggtacgtggatggcgtggaggtgcacaatgccaagaccaagccaagagaggagcagtttaactctacatacagggtggtgagcgtgctgaccgtgctgcaccaggattggctcaacggcaaggagtataagtgcaaggtgtccaataagggcctgccctcctctatcgagaagacaatctctaaggctaagggccagccaagagagcctcaggtgtacaccctgcctccaagccaggaggagatgacaaagaaccaggtgtccctgacatgtctggtgaagggcttctatccctccgacatcgccgtggagtgggagtctaatggccagcctgagaacaattacaagaccacaccccctgtgctggactctgatggcagcttctttctgtattccaggctgaccgtggataagtctcggtggcaggagggcaacgtgttcagctgctctgtgatgcacgaagccctgcataatcactatactcagaaaagtctgtcactgtcactgggaaagtgataa

SEQ ID NO: 47 - protein, 445 aa, Artificial Sequence
  Humanized antibody, 1G1-h70 heavy chain amino acids
QVQLVQSGAEVKKPGASVKVSCKASGYTFTGYWMHWVRQAPGQGLEWIGMIHPNSDTTTYNEKFKNRVTMTRDTSISTAYMELSRLRSDDTAVYYCAGTDQAAWFAFWGQGTTVTVSSASTKGPSVFPLAPCSRSTSESTAALGCLVKDYFPEPVTVSWNSGALTSGVHTFPAVLQSSGLYSLSSVVTVPSSSLGTKTYTCNVDHKPSNTKVDKRVESKYGPPCPSCPAPEFLGGPSVFLFPPKPKDTLMISRTPEVTCVVVDVSQEDPEVQFNWYVDGVEVHNAKTKPREEQFNSTYRVVSVLTVLHQDWLNGKEYKCKVSNKGLPSSIEKTISKAKGQPREPQVYTLPPSQEEMTKNQVSLTCLVKGFYPSDIAVEWESNGQPENNYKTTPPVLDSDGSFFLYSRLTVDKSRWQEGNVFSCSVMHEALHNHYTQKSLSLSLGK

SEQ ID NO: 48 - DNA, 663 bp, Artificial Sequence
  Humanized antibody, 1G1-h61 light chain nucleotides
gatatcgttatgacccagacccctctgagcctgtccgtgaccccaggccaacctgcctctatcagctgtagaagcagccagaacatcgtgcacagcaacggcgacacctacctggaatggtatctgcagaaacctggacagagccccaagctgctgatctacaaggtgtccaagcggttttccggcgtgcctgatagattcagcggatctggcagcggcacagacttcaccctgaagatttctagagtggaggccgaggacgtgggcgtctactactgcttccagggcagccacgtgccctggacattcggcggcggaacaaaggtggaaatcaagaggacagtggccgccccaagcgtgttcatctttcccccttccgacgagcagctgaagtctggcaccgccagcgtggtgtgcctgctgaacaacttctaccctcgggaggccaaggtccagtggaaggtggataacgccctgcagtctggcaatagccaggagtccgtgaccgagcaggactctaaggatagcacatattccctgtctagcaccctgacactgagcaaggccgattacgagaagcacaaggtgtatgcctgtgaagtcacccatcaggggctgtcatcacccgtcactaagtcattcaatcgcggagaatgctgataa

SEQ ID NO: 49 - protein, 219 aa, Artificial Sequence
  Humanized antibody, 1G1-h61 light chain amino acids
DIVMTQTPLSLSVTPGQPASISCRSSQNIVHSNGDTYLEWYLQKPGQSPKLLIYKVSKRFSGVPDRFSGSGSGTDFTLKISRVEAEDVGVYYCFQGSHVPWTFGGGTKVEIKRTVAAPSVFIFPPSDEQLKSGTASVVCLLNNFYPREAKVQWKVDNALQSGNSQESVTEQDSKDSTYSLSSTLTLSKADYEKHKVYACEVTHQGLSSPVTKSFNRGEC

SEQ ID NO: 50 - DNA, 663 bp, Artificial Sequence
  Humanized antibody, 1G1-h68 light chain nucleotides
gatatcgttatgacccagacccctctgagcctgtccgtgaccccaggccaacctgcctctatcagctgtagaagcagccagaacatcgtgcacagcaacggcgacacctacctggaatggtatctgcagaaacctggacagagcccccagctgctgatctacaaggtgtccaagcggttttccggcgtgcctgatagattcagcggatctggcagcggcacagacttcaccctgaagatttctagagtggaggccgaggacgtgggcgtctactactgcttccagggcagccacgtgccctggacattcggcggcggaacaaaggtggaaatcaagaggacagtggccgccccaagcgtgttcatctttcccccttccgacgagcagctgaagtctggcaccgccagcgtggtgtgcctgctgaacaacttctaccctcgggaggccaaggtccagtggaaggtggataacgccctgcagtctggcaatagccaggagtccgtgaccgagcaggactctaaggatagcacatattccctgtctagcaccctgacactgagcaaggccgattacgagaagcacaaggtgtatgcctgtgaagtcacccatcaggggctgtcatcacccgtcactaagtcattcaatcgcggagaatgctgataa

SEQ ID NO: 51 - protein, 219 aa, Artificial Sequence
  Humanized antibody, 1G1-h68 light chain amino acids
DIVMTQTPLSLSVTPGQPASISCRSSQNIVHSNGDTYLEWYLQKPGQSPQLLIYKVSKRFSGVPDRFSGSGSGTDFTLKISRVEAEDVGVYYCFQGSHVPWTFGGGTKVEIKRTVAAPSVFIFPPSDEQLKSGTASVVCLLNNFYPREAKVQWKVDNALQSGNSQESVTEQDSKDSTYSLSSTLTLSKADYEKHKVYACEVTHQGLSSPVTKSFNRGEC

SEQ ID NO: 52 - DNA, 663 bp, Artificial Sequence
  Humanized antibody, 1G1-h70 light chain nucleotides
gatatcgttatgacccagacccctctgagcctgtccgtgaccccaggccaacctgcctctatcagctgtagaagcagccagaacatcgtgcacagccagggcgacacctacctggaatggtatctgcagaaacctggacagagcccccagctgctgatctacaaggtgtccaagcggttttccggcgtgcctgatagattcagcggatctggcagcggcacagacttcaccctgaagatttctagagtggaggccgaggacgtgggcgtctactactgcttccagggcagccacgtgccctggacattcggcggcggaacaaaggtggaaatcaagaggacagtggccgccccaagcgtgttcatctttcccccttccgacgagcagctgaagtctggcaccgccagcgtggtgtgcctgctgaacaacttctaccctcgggaggccaaggtccagtggaaggtggataacgccctgcagtctggcaatagccaggagtccgtgaccgagcaggactctaaggatagcacatattccctgtctagcaccctgacactgagcaaggccgattacgagaagcacaaggtgtatgcctgtgaagtcacccatcaggggctgtcatcacccgtcactaagtcattcaatcgcggagaatgctgataa

SEQ ID NO: 53 - protein, 219 aa, Artificial Sequence
  Humanized antibody, 1G1-h70 light chain amino acids
DIVMTQTPLSLSVTPGQPASISCRSSQNIVHSQGDTYLEWYLQKPGQSPQLLIYKVSKRFSGVPDRFSGSGSGTDFTLKISRVEAEDVGVYYCFQGSHVPWTFGGGTKVEIKRTVAAPSVFIFPPSDEQLKSGTASVVCLLNNFYPREAKVQWKVDNALQSGNSQESVTEQDSKDSTYSLSSTLTLSKADYEKHKVYACEVTHQGLSSPVTKSFNRGEC

SEQ ID NO: 54 - protein, 118 aa, Artificial Sequence
  Humanized antibody, 1G1-h61 VH amino acids
QVQLVQSGAEVKKPGASVKVSCKASGYTFTGYWMHWVRQAPGQGLEWMGMIHPNSDTTTYNEKFKNRVTMTRDTSISTAYMELSRLRSDDTAVYYCAGTDQAAWFAFWGQGTTVTVSS

SEQ ID NO: 55 - protein, 112 aa, Artificial Sequence
  Humanized antibody, 1G1-h61 VL amino acids
DIVMTQTPLSLSVTPGQPASISCRSSQNIVHSNGDTYLEWYLQKPGQSPKLLIYKVSKRFSGVPDRFSGSGSGTDFTLKISRVEAEDVGVYYCFQGSHVPWTFGGGTKVEIK

SEQ ID NO: 56 - protein, 118 aa, Artificial Sequence
  Humanized antibody, 1G1-h68 VH amino acids
QVQLVQSGAEVKKPGASVKVSCKASGYTFTGYWMHWVRQAPGQGLEWIGMIHPNSDTTTYNEKFKNRVTMTRDTSISTAYMELSRLRSDDTAVYYCTGTDQAAWFAFWGQGTTVTVSS

SEQ ID NO: 57 - protein, 112 aa, Artificial Sequence
  Humanized antibody, 1G1-h68 VL amino acids
DIVMTQTPLSLSVTPGQPASISCRSSQNIVHSNGDTYLEWYLQKPGQSPQLLIYKVSKRFSGVPDRFSGSGSGTDFTLKISRVEAEDVGVYYCFQGSHVPWTFGGGTKVEIK

SEQ ID NO: 58 - protein, 118 aa, Artificial Sequence
  Humanized antibody, 1G1-h70 VH amino acids
QVQLVQSGAEVKKPGASVKVSCKASGYTFTGYWMHWVRQAPGQGLEWIGMIHPNSDTTTYNEKFKNRVTMTRDTSISTAYMELSRLRSDDTAVYYCAGTDQAAWFAFWGQGTTVTVSS

SEQ ID NO: 59 - protein, 112 aa, Artificial Sequence
  Humanized antibody, 1G1-h70 VL amino acids
DIVMTQTPLSLSVTPGQPASISCRSSQNIVHSQGDTYLEWYLQKPGQSPQLLIYKVSKRFSGVPDRFSGSGSGTDFTLKISRVEAEDVGVYYCFQGSHVPWTFGGGTKVEIK

SEQ ID NO: 60 - protein, 16 aa, Artificial Sequence
  LCDR1 amino acids
RSSQNIVHSQGDTYLE

SEQ ID NO: 61 - DNA, 48 bp, Artificial Sequence
  LCDR1 nucleotides
agaagcagccagaacatcgtgcacagccagggcgacacctacctggaa

SEQ ID NO: 62 - protein, 288 aa, Artificial Sequence
  Human PD-1 protein, full amino acids
MQIPQAPWPVVWAVLQLGWRPGWFLDSPDRPWNPPTFSPALLVVTEGDNATFTCSFSNTSESFVLNWYRMSPSNQTDKLAAFPEDRSQPGQDCRFRVTQLPNGRDFHMSVVRARRNDSGTYLCGAISLAPKAQIKESLRAELRVTERRAEVPTAHPSPSPRPAGQFQTLVVGVVGGLLGSLVLLVWVLAVICSRAARGTIGARRTGQPLKEDPSAVPVFSVDYGELDFQWREKTPEPPVPCVPEQTEYATIVFPSGMGTSSPARRGSADGPRSAQPLRPEDGHCSWPL

SEQ ID NO: 63 - protein, 17 aa, Artificial Sequence
  HCDR2 aa
MIHPNSDTTVYNEKFKN

SEQ ID NO: 64 - protein, 17 aa, Artificial Sequence
  HCDR2 aa
MIHPNSDTTIYNEKFKN

SEQ ID NO: 65 - protein, 17 aa, Artificial Sequence
  HCDR2 aa
MIHPNSDTTTYNWKFKN

SEQ ID NO: 66 - protein, 17 aa, Artificial Sequence
  HCDR2 aa
MIHPNSDTTVYNWKFKN

SEQ ID NO: 67 - protein, 17 aa, Artificial Sequence
  HCDR2 aa
MIHPNSDTTIYNWKFKN

SEQ ID NO: 68 - protein, 9 aa, Artificial Sequence
  HCDR3 aa
TDQEAWFAF

SEQ ID NO: 69 - protein, 9 aa, Artificial Sequence
  HCDR3 aa
TDQAAWAAF

SEQ ID NO: 70 - protein, 9 aa, Artificial Sequence
  HCDR3 aa
TDQAAWMAF

SEQ ID NO: 71 - protein, 9 aa, Artificial Sequence
  HCDR3 aa
TDQAAWHAF

SEQ ID NO: 72 - protein, 9 aa, Artificial Sequence
  HCDR3 aa
TDQAAWFGF

SEQ ID NO: 73 - protein, 9 aa, Artificial Sequence
  HCDR3 aa
TDQEAWAAF

SEQ ID NO: 74 - protein, 9 aa, Artificial Sequence
  HCDR3 aa
TDQEAWMAF

SEQ ID NO: 75 - protein, 9 aa, Artificial Sequence
  HCDR3 aa
TDQEAWHAF

SEQ ID NO: 76 - protein, 9 aa, Artificial Sequence
  HCDR3 aa
TDQEAWFGF

SEQ ID NO: 77 - protein, 9 aa, Artificial Sequence
  HCDR3 aa
TDQAAWAGF

SEQ ID NO: 78 - protein, 9 aa, Artificial Sequence
  HCDR3 aa
TDQAAWMGF

SEQ ID NO: 79 - protein, 9 aa, Artificial Sequence
  HCDR3 aa
TDQAAWHGF

SEQ ID NO: 80 - protein, 9 aa, Artificial Sequence
  HCDR3 aa
TDQEAWAGF

SEQ ID NO: 81 - protein, 9 aa, Artificial Sequence
  HCDR3 aa
TDQEAWMGF

SEQ ID NO: 82 - protein, 9 aa, Artificial Sequence
  HCDR3 aa
TDQEAWHGF

SEQ ID NO: 83 - protein, 16 aa, Artificial Sequence
  LCDR1 aa
RSSQNIVRSNGDTYLE

SEQ ID NO: 84 - protein, 16 aa, Artificial Sequence
  LCDR1 aa
RSSQNIVRSQGDTYLE